European Patent Specification EP 3 522 902 B1, published September 3, 2025. Title: USE OF AHR AGONIST FOR THE PREVENTIVE OR CURATIVE TREATMENT OF METABOLIC SYNDROME AND THE ASSOCIATED DISORDERS. Applicant: INRA et al. The sequence listing filed with the application follows.

SEQUENCE LISTING (8 sequences)

SEQ ID NO: 1 - DNA, 20 bp, artificial sequence
  primer
aactttggcattgtggaagg

SEQ ID NO: 2 - DNA, 20 bp, artificial sequence
  primer
acacattgggggtaggaaca

SEQ ID NO: 3 - DNA, 20 bp, artificial sequence
  primer
catgcaggaggtggtacctt

SEQ ID NO: 4 - DNA, 20 bp, artificial sequence
  primer
cagacgcaagcatttctcag

SEQ ID NO: 5 - DNA, 22 bp, artificial sequence
  primer
ttcctgtcctccatgatcaaaa

SEQ ID NO: 6 - DNA, 21 bp, artificial sequence
  primer
catccacctctgttgggttca

SEQ ID NO: 7 - DNA, 21 bp, artificial sequence
  primer
atgctgctctcctgcctgatg

SEQ ID NO: 8 - DNA, 24 bp, artificial sequence
  primer
ctaatgcgtgcggagggtatattc